European Patent Specification EP 4 138 887 B1, published August 19, 2026. Title: COMPOSITIONS AND METHODS OF TREATING CANCER WITH CHIMERIC ANTIGEN RECEPTORS. Applicant: ASTRAZENECA AB. The sequence listing filed with the application follows.

SEQUENCE LISTING (48 sequences)

SEQ ID NO: 1 - protein, 241 aa, Artificial Sequence
  source: /note="Description of Artificial Sequence: Synthetic polypeptide"
EVQLLESGGGLVQPGGSLRLSCAASGFTFSSYAMSWVRQAPGKGLEWVSAISGSGGSTYYADSVKGRFTISRDNSKNTLYLQMNSLRAEDTAVYYCARGKRYFDYWGQGTMVTVSSGGGGSGGGGSGGGGSSYELTQPPSASGTPGQRVTISCSGGSSNIGSNTVNWFRQLPGTAPKLLVYFNNQRPSGVPDRFSGSKSGTSASLAIGGLQSDDEADYYCVAWDDSLNAPVFGGGTKVTVL

SEQ ID NO: 2 - protein, 241 aa, Artificial Sequence
  source: /note="Description of Artificial Sequence: Synthetic polypeptide"
EVQLLESGGGLVQPGGSLRLSCAASGFTFSSYAMSWVRQAPGKGLEWVSAISGSGGSTYYADSVKGRFTISRDNSKNTLYLQMNSLRAEDTAVYYCAKGKRYFDYWGQGTMVTVSSGGGGSGGGGSGGGGSQSVLTQPPSASGTPGQRVTISCSGGSSDIGSNTVNWYQQLPGTAPKLLIYYNNQRPSGVPDRFSGSKSGTSASLAISGLQSEDEADYYCATWDDRMYSPVFGGGTKLTVL

SEQ ID NO: 3 - protein, 460 aa, Artificial Sequence
  source: /note="Description of Artificial Sequence: Synthetic polypeptide"
MLLLVTSLLLCELPHPAFLLIPGVHSEVQLLESGGGLVQPGGSLRLSCAASGFTFSSYAMSWVRQAPGKGLEWVSAISGSGGSTYYADSVKGRFTISRDNSKNTLYLQMNSLRAEDTAVYYCARGKRYFDYWGQGTMVTVSSGGGGSGGGGSGGGGSSYELTQPPSASGTPGQRVTISCSGGSSNIGSNTVNWFRQLPGTAPKLLVYFNNQRPSGVPDRFSGSKSGTSASLAIGGLQSDDEADYYCVAWDDSLNAPVFGGGTKVTVLESKYGPPCPPCPFWVLVVVGGVLACYSLLVTVAFIIFWVKRGRKKLLYIFKQPFMRPVQTTQEEDGCSCRFPEEEEGGCELRVKFSRSADAPAYQQGQNQLYNELNLGRREEYDVLDKRRGRDPEMGGKPRRKNPQEGLYNELQKDKMAEAYSEIGMKGERRRGKGHDGLYQGLSTATKDTYDALHMQALPPR

SEQ ID NO: 4 - protein, 318 aa, Artificial Sequence
  source: /note="Description of Artificial Sequence: Synthetic polypeptide"
MLLLVTSLLLCELPHPAFLLIPGVHSEVQLLESGGGLVQPGGSLRLSCAASGFTFSSYAMSWVRQAPGKGLEWVSAISGSGGSTYYADSVKGRFTISRDNSKNTLYLQMNSLRAEDTAVYYCARGKRYFDYWGQGTMVTVSSGGGGSGGGGSGGGGSSYELTQPPSASGTPGQRVTISCSGGSSNIGSNTVNWFRQLPGTAPKLLVYFNNQRPSGVPDRFSGSKSGTSASLAIGGLQSDDEADYYCVAWDDSLNAPVFGGGTKVTVLESKYGPPCPPCPFWVLVVVGGVLACYSLLVTVAFIIFWVRVKFSRSADAPA

SEQ ID NO: 5 - protein, 459 aa, Artificial Sequence
  source: /note="Description of Artificial Sequence: Synthetic polypeptide"
MLLLVTSLLLCELPHPAFLLIPGVHSEVQLLESGGGLVQPGGSLRLSCAASGFTFSSYAMSWVRQAPGKGLEWVSAISGSGGSTYYADSVKGRFTISRDNSKNTLYLQMNSLRAEDTAVYYCARGKRYFDYWGQGTMVTVSSGGGGSGGGGSGGGGSSYELTQPPSASGTPGQRVTISCSGGSSNIGSNTVNWFRQLPGTAPKLLVYFNNQRPSGVPDRFSGSKSGTSASLAIGGLQSDDEADYYCVAWDDSLNAPVFGGGTKVTVLESKYGPPCPPCPFWVLVVVGGVLACYSLLVTVAFIIFWVRSKRSRLLHSDYMNMTPRRPGPTRKHYQPYAPPRDFAAYRSRVKFSRSADAPAYQQGQNQLYNELNLGRREEYDVLDKRRGRDPEMGGKPRRKNPQEGLYNELQKDKMAEAYSEIGMKGERRRGKGHDGLYQGLSTATKDTYDALHMQALPPR

SEQ ID NO: 6 - protein, 501 aa, Artificial Sequence
  source: /note="Description of Artificial Sequence: Synthetic polypeptide"
MLLLVTSLLLCELPHPAFLLIPGVHSEVQLLESGGGLVQPGGSLRLSCAASGFTFSSYAMSWVRQAPGKGLEWVSAISGSGGSTYYADSVKGRFTISRDNSKNTLYLQMNSLRAEDTAVYYCARGKRYFDYWGQGTMVTVSSGGGGSGGGGSGGGGSSYELTQPPSASGTPGQRVTISCSGGSSNIGSNTVNWFRQLPGTAPKLLVYFNNQRPSGVPDRFSGSKSGTSASLAIGGLQSDDEADYYCVAWDDSLNAPVFGGGTKVTVLESKYGPPCPPCPFWVLVVVGGVLACYSLLVTVAFIIFWVRSKRSRLLHSDYMNMTPRRPGPTRKHYQPYAPPRDFAAYRSKRGRKKLLYIFKQPFMRPVQTTQEEDGCSCRFPEEEEGGCELRVKFSRSADAPAYQQGQNQLYNELNLGRREEYDVLDKRRGRDPEMGGKPRRKNPQEGLYNELQKDKMAEAYSEIGMKGERRRGKGHDGLYQGLSTATKDTYDALHMQALPPR

SEQ ID NO: 7 - protein, 456 aa, Artificial Sequence
  source: /note="Description of Artificial Sequence: Synthetic polypeptide"
MLLLVTSLLLCELPHPAFLLIPEVQLLESGGGLVQPGGSLRLSCAASGFTFSSYAMSWVRQAPGKGLEWVSAISGSGGSTYYADSVKGRFTISRDNSKNTLYLQMNSLRAEDTAVYYCAKGKRYFDYWGQGTMVTVSSGGGGSGGGGSGGGGSQSVLTQPPSASGTPGQRVTISCSGGSSDIGSNTVNWYQQLPGTAPKLLIYYNNQRPSGVPDRFSGSKSGTSASLAISGLQSEDEADYYCATWDDRMYSPVFGGGTKLTVLESKYGPPCPPCPFWVLVVVGGVLACYSLLVTVAFIIFWVKRGRKKLLYIFKQPFMRPVQTTQEEDGCSCRFPEEEEGGCELRVKFSRSADAPAYQQGQNQLYNELNLGRREEYDVLDKRRGRDPEMGGKPRRKNPQEGLYNELQKDKMAEAYSEIGMKGERRRGKGHDGLYQGLSTATKDTYDALHMQALPPR

SEQ ID NO: 8 - protein, 314 aa, Artificial Sequence
  source: /note="Description of Artificial Sequence: Synthetic polypeptide"
MLLLVTSLLLCELPHPAFLLIPEVQLLESGGGLVQPGGSLRLSCAASGFTFSSYAMSWVRQAPGKGLEWVSAISGSGGSTYYADSVKGRFTISRDNSKNTLYLQMNSLRAEDTAVYYCAKGKRYFDYWGQGTMVTVSSGGGGSGGGGSGGGGSQSVLTQPPSASGTPGQRVTISCSGGSSDIGSNTVNWYQQLPGTAPKLLIYYNNQRPSGVPDRFSGSKSGTSASLAISGLQSEDEADYYCATWDDRMYSPVFGGGTKLTVLESKYGPPCPPCPFWVLVVVGGVLACYSLLVTVAFIIFWVRVKFSRSADAPA

SEQ ID NO: 9 - protein, 455 aa, Artificial Sequence
  source: /note="Description of Artificial Sequence: Synthetic polypeptide"
MLLLVTSLLLCELPHPAFLLIPEVQLLESGGGLVQPGGSLRLSCAASGFTFSSYAMSWVRQAPGKGLEWVSAISGSGGSTYYADSVKGRFTISRDNSKNTLYLQMNSLRAEDTAVYYCAKGKRYFDYWGQGTMVTVSSGGGGSGGGGSGGGGSQSVLTQPPSASGTPGQRVTISCSGGSSDIGSNTVNWYQQLPGTAPKLLIYYNNQRPSGVPDRFSGSKSGTSASLAISGLQSEDEADYYCATWDDRMYSPVFGGGTKLTVLESKYGPPCPPCPFWVLVVVGGVLACYSLLVTVAFIIFWVRSKRSRLLHSDYMNMTPRRPGPTRKHYQPYAPPRDFAAYRSRVKFSRSADAPAYQQGQNQLYNELNLGRREEYDVLDKRRGRDPEMGGKPRRKNPQEGLYNELQKDKMAEAYSEIGMKGERRRGKGHDGLYQGLSTATKDTYDALHMQALPPR

SEQ ID NO: 10 - protein, 497 aa, Artificial Sequence
  source: /note="Description of Artificial Sequence: Synthetic polypeptide"
MLLLVTSLLLCELPHPAFLLIPEVQLLESGGGLVQPGGSLRLSCAASGFTFSSYAMSWVRQAPGKGLEWVSAISGSGGSTYYADSVKGRFTISRDNSKNTLYLQMNSLRAEDTAVYYCAKGKRYFDYWGQGTMVTVSSGGGGSGGGGSGGGGSQSVLTQPPSASGTPGQRVTISCSGGSSDIGSNTVNWYQQLPGTAPKLLIYYNNQRPSGVPDRFSGSKSGTSASLAISGLQSEDEADYYCATWDDRMYSPVFGGGTKLTVLESKYGPPCPPCPFWVLVVVGGVLACYSLLVTVAFIIFWVRSKRSRLLHSDYMNMTPRRPGPTRKHYQPYAPPRDFAAYRSKRGRKKLLYIFKQPFMRPVQTTQEEDGCSCRFPEEEEGGCELRVKFSRSADAPAYQQGQNQLYNELNLGRREEYDVLDKRRGRDPEMGGKPRRKNPQEGLYNELQKDKMAEAYSEIGMKGERRRGKGHDGLYQGLSTATKDTYDALHMQALPPR

SEQ ID NO: 11 - DNA, 1383 bp, Artificial Sequence
  source: /note="Description of Artificial Sequence: Synthetic polynucleotide"
atgctgctgctggtgacaagcctgctgctgtgcgaactgccccatcccgccttcctgctgattcctggtgtacactccgaggtgcagctgttggagtctgggggaggcttggtacagcctggggggtccctgagactctcctgtgcagcctctggattcacctttagcagctatgccatgagctgggtccgccaggctccagggaaggggctggagtgggtctcagctattagtggtagtggtggtagcacatactacgcagactccgtgaagggccggttcaccatctccagagacaattccaagaacacgctgtatctgcaaatgaacagcctgagagccgaggacacggccgtgtattactgtgcgagaggaaagcgatactttgactactggggccaggggacaatggtcaccgtctcgagtggtggggggggcagcggtggtggaggctctggtggaggagggagctcctatgagctgactcagccaccctcagcgtctgggacccccgggcagagggtcaccatctcttgttctggaggcagctccaacatcggaagtaatactgtaaactggttccggcagctcccaggaacggcccccaaactcctcgtttattttaataatcagcgaccctcaggggtccctgaccgattctctggctccaagtctggcacctcggcctccctggccatcggtgggctccagtctgacgatgaggctgactattactgtgtagcatgggatgactctctgaatgctccggtgttcggcggagggaccaaggtcaccgtcctagagagcaaatatggaccaccatgccctccatgtcctttttgggtcctggtggtcgtgggaggcgtgctggcatgttattctctgctggtcacagtggctttcatcatcttctgggtcaagcgaggccggaagaaactgctgtacatcttcaaacagccttttatgcgcccagtgcagacaactcaggaggaagacggctgctcttgtcggttccccgaggaagaggaagggggatgtgagctgcgcgtgaagttttctcgaagtgccgatgctcctgcatatcagcagggacagaaccagctgtacaacgagctgaatctgggccggagagaggaatacgacgtgctggataagaggcgcggcagagacccagaaatgggcgggaagccacgacggaaaaacccccaggaggggctgtataatgaactgcagaaggacaaaatggccgaggcttacagcgaaatcgggatgaagggagagagaaggcgcggaaaaggccacgatggactgtatcagggcctgagcactgccaccaaggacacctacgatgctctgcacatgcaggcactgccacccaggtga

SEQ ID NO: 12 - DNA, 957 bp, Artificial Sequence
  source: /note="Description of Artificial Sequence: Synthetic polynucleotide"
atgctgctgctggtgacaagcctgctgctgtgcgaactgccccatcccgccttcctgctgattcctggtgtacactccgaggtgcagctgttggagtctgggggaggcttggtacagcctggggggtccctgagactctcctgtgcagcctctggattcacctttagcagctatgccatgagctgggtccgccaggctccagggaaggggctggagtgggtctcagctattagtggtagtggtggtagcacatactacgcagactccgtgaagggccggttcaccatctccagagacaattccaagaacacgctgtatctgcaaatgaacagcctgagagccgaggacacggccgtgtattactgtgcgagaggaaagcgatactttgactactggggccaggggacaatggtcaccgtctcgagtggtggggggggcagcggtggtggaggctctggtggaggagggagctcctatgagctgactcagccaccctcagcgtctgggacccccgggcagagggtcaccatctcttgttctggaggcagctccaacatcggaagtaatactgtaaactggttccggcagctcccaggaacggcccccaaactcctcgtttattttaataatcagcgaccctcaggggtccctgaccgattctctggctccaagtctggcacctcggcctccctggccatcggtgggctccagtctgacgatgaggctgactattactgtgtagcatgggatgactctctgaatgctccggtgttcggcggagggaccaaggtcaccgtcctagagagcaaatatggaccaccatgccctccatgtcctttttgggtcctggtggtcgtgggaggcgtgctggcatgttattctctgctggtcacagtggctttcatcatcttctgggtccgcgtgaagttttctcgaagtgccgatgctcctgcatga

SEQ ID NO: 13 - DNA, 1380 bp, Artificial Sequence
  source: /note="Description of Artificial Sequence: Synthetic polynucleotide"
atgctgctgctggtgacaagcctgctgctgtgcgaactgccccatcccgccttcctgctgattcctggtgtacactccgaggtgcagctgttggagtctgggggaggcttggtacagcctggggggtccctgagactctcctgtgcagcctctggattcacctttagcagctatgccatgagctgggtccgccaggctccagggaaggggctggagtgggtctcagctattagtggtagtggtggtagcacatactacgcagactccgtgaagggccggttcaccatctccagagacaattccaagaacacgctgtatctgcaaatgaacagcctgagagccgaggacacggccgtgtattactgtgcgagaggaaagcgatactttgactactggggccaggggacaatggtcaccgtctcgagtggtggggggggcagcggtggtggaggctctggtggaggagggagctcctatgagctgactcagccaccctcagcgtctgggacccccgggcagagggtcaccatctcttgttctggaggcagctccaacatcggaagtaatactgtaaactggttccggcagctcccaggaacggcccccaaactcctcgtttattttaataatcagcgaccctcaggggtccctgaccgattctctggctccaagtctggcacctcggcctccctggccatcggtgggctccagtctgacgatgaggctgactattactgtgtagcatgggatgactctctgaatgctccggtgttcggcggagggaccaaggtcaccgtcctagagagcaaatatggaccaccatgccctccatgtcctttttgggtcctggtggtcgtgggaggcgtgctggcatgttattccctgctggtcactgtggccttcatcatcttctgggtgcggagcaagcggagccggctgctgcactctgactacatgaacatgactccacggagacccggccctacccggaaacattatcagccctacgccccacccagagattttgccgcttataggtccagggtgaagttttctcgcagtgcagatgcccctgcttatcagcagggacagaatcagctgtacaacgagctgaatctgggcaggcgcgaggaatacgacgtgctggataagcgacggggcagagaccccgaaatgggagggaagcccagaaggaaaaaccctcaggaggggctgtataatgaactgcagaaggacaaaatggcagaggcctacagtgaaatcgggatgaagggagagcgccgacggggaaaaggccacgatggactgtatcagggcctgtctactgccaccaaggacacctacgatgccctgcacatgcaggctctgcctccacgctga

SEQ ID NO: 14 - DNA, 1506 bp, Artificial Sequence
  source: /note="Description of Artificial Sequence: Synthetic polynucleotide"
atgctgctgctggtgacaagcctgctgctgtgcgaactgccccatcccgccttcctgctgattcctggtgtacactccgaggtgcagctgttggagtctgggggaggcttggtacagcctggggggtccctgagactctcctgtgcagcctctggattcacctttagcagctatgccatgagctgggtccgccaggctccagggaaggggctggagtgggtctcagctattagtggtagtggtggtagcacatactacgcagactccgtgaagggccggttcaccatctccagagacaattccaagaacacgctgtatctgcaaatgaacagcctgagagccgaggacacggccgtgtattactgtgcgagaggaaagcgatactttgactactggggccaggggacaatggtcaccgtctcgagtggtggggggggcagcggtggtggaggctctggtggaggagggagctcctatgagctgactcagccaccctcagcgtctgggacccccgggcagagggtcaccatctcttgttctggaggcagctccaacatcggaagtaatactgtaaactggttccggcagctcccaggaacggcccccaaactcctcgtttattttaataatcagcgaccctcaggggtccctgaccgattctctggctccaagtctggcacctcggcctccctggccatcggtgggctccagtctgacgatgaggctgactattactgtgtagcatgggatgactctctgaatgctccggtgttcggcggagggaccaaggtcaccgtcctagagagcaaatatggaccaccatgccctccatgtcctttttgggtcctggtggtcgtgggaggcgtgctggcatgttattccctgctggtcactgtggccttcatcatcttctgggtgcggagcaagcggagccggctgctgcactctgactacatgaacatgactccacggagacccggccctacccggaaacattatcagccctacgccccacccagagattttgccgcttataggtccaagcgcggccgaaagaaactgctgtacatcttcaaacagcccttcatgagacccgtccagacaactcaggaggaagacggctgcagctgtaggttccccgaggaagaggaagggggatgtgagctgagggtgaagttttctcgcagtgcagatgcccctgcttatcagcagggacagaatcagctgtacaacgagctgaatctgggcaggcgcgaggaatacgacgtgctggataagcgacggggcagagaccccgaaatgggagggaagcccagaaggaaaaaccctcaggaggggctgtataatgaactgcagaaggacaaaatggcagaggcctacagtgaaatcgggatgaagggagagcgccgacggggaaaaggccacgatggactgtatcagggcctgtctactgccaccaaggacacctacgatgccctgcacatgcaggctctgcctccacgctga

SEQ ID NO: 15 - DNA, 1371 bp, Artificial Sequence
  source: /note="Description of Artificial Sequence: Synthetic polynucleotide"
atgctgctgctggtgacaagcctgctgctgtgcgaactgccccatcccgccttcctgctgattcctgaggtccagctgctggagagcggaggaggactggtgcagcctggaggaagtctgcgactgtcatgcgccgctagcggcttcaccttcagctcctatgcaatgagctgggtgcgacaggcaccaggcaaggggctggagtgggtctccgctatctccggctctggaggctctacttactatgcagacagtgtgaaggggcggttcacaatctccagagataactctaagaacactctgtacctgcagatgaactctctgagagctgaggacaccgcagtgtactattgcgccaagggcaaaaggtactttgattattggggacagggcactatggtgaccgtctctagtggaggaggaggaagcggaggaggaggatccggcggaggaggcagtcagtcagtgctgacacagccacctagcgcctccggaaccccaggacagcgggtcacaatctcttgtagtgggggatcaagcgacattgggagcaacaccgtgaattggtatcagcagctgcctggaacagctccaaagctgctgatctactataacaatcagaggccctccggcgtccctgatcgcttctcaggcagcaaatccgggacttctgcaagtctggccattagtggcctgcagtcagaggacgaagccgattactattgtgctacctgggacgataggatgtactctcccgtgttcggcgggggaacaaagctgactgtcctggagagcaaatatggaccaccatgccctccatgtcctttttgggtcctggtggtcgtgggaggcgtgctggcatgttattctctgctggtcacagtggctttcatcatcttctgggtcaagcgaggccggaagaaactgctgtacatcttcaaacagccttttatgcgcccagtgcagacaactcaggaggaagacggctgctcttgtcggttccccgaggaagaggaagggggatgtgagctgcgcgtgaagttttctcgaagtgccgatgctcctgcatatcagcagggacagaaccagctgtacaacgagctgaatctgggccggagagaggaatacgacgtgctggataagaggcgcggcagagacccagaaatgggcgggaagccacgacggaaaaacccccaggaggggctgtataatgaactgcagaaggacaaaatggccgaggcttacagcgaaatcgggatgaagggagagagaaggcgcggaaaaggccacgatggactgtatcagggcctgagcactgccaccaaggacacctacgatgctctgcacatgcaggcactgccacccaggtga

SEQ ID NO: 16 - DNA, 945 bp, Artificial Sequence
  source: /note="Description of Artificial Sequence: Synthetic polynucleotide"
atgctgctgctggtgacaagcctgctgctgtgcgaactgccccatcccgccttcctgctgattcctgaggtccagctgctggagagcggaggaggactggtgcagcctggaggaagtctgcgactgtcatgcgccgctagcggcttcaccttcagctcctatgcaatgagctgggtgcgacaggcaccaggcaaggggctggagtgggtctccgctatctccggctctggaggctctacttactatgcagacagtgtgaaggggcggttcacaatctccagagataactctaagaacactctgtacctgcagatgaactctctgagagctgaggacaccgcagtgtactattgcgccaagggcaaaaggtactttgattattggggacagggcactatggtgaccgtctctagtggaggaggaggaagcggaggaggaggatccggcggaggaggcagtcagtcagtgctgacacagccacctagcgcctccggaaccccaggacagcgggtcacaatctcttgtagtgggggatcaagcgacattgggagcaacaccgtgaattggtatcagcagctgcctggaacagctccaaagctgctgatctactataacaatcagaggccctccggcgtccctgatcgcttctcaggcagcaaatccgggacttctgcaagtctggccattagtggcctgcagtcagaggacgaagccgattactattgtgctacctgggacgataggatgtactctcccgtgttcggcgggggaacaaagctgactgtcctggagagcaaatatggaccaccatgccctccatgtcctttttgggtcctggtggtcgtgggaggcgtgctggcatgttactccctgctggtcactgtggccttcatcatcttctgggtgcgggtgaagttttctcgcagtgccgacgctcccgcatga

SEQ ID NO: 17 - DNA, 1368 bp, Artificial Sequence
  source: /note="Description of Artificial Sequence: Synthetic polynucleotide"
atgctgctgctggtgacaagcctgctgctgtgcgaactgccccatcccgccttcctgctgattcctgaggtccagctgctggagagcggaggaggactggtgcagcctggaggaagtctgcgactgtcatgcgccgctagcggcttcaccttcagctcctatgcaatgagctgggtgcgacaggcaccaggcaaggggctggagtgggtctccgctatctccggctctggaggctctacttactatgcagacagtgtgaaggggcggttcacaatctccagagataactctaagaacactctgtacctgcagatgaactctctgagagctgaggacaccgcagtgtactattgcgccaagggcaaaaggtactttgattattggggacagggcactatggtgaccgtctctagtggaggaggaggaagcggaggaggaggatccggcggaggaggcagtcagtcagtgctgacacagccacctagcgcctccggaaccccaggacagcgggtcacaatctcttgtagtgggggatcaagcgacattgggagcaacaccgtgaattggtatcagcagctgcctggaacagctccaaagctgctgatctactataacaatcagaggccctccggcgtccctgatcgcttctcaggcagcaaatccgggacttctgcaagtctggccattagtggcctgcagtcagaggacgaagccgattactattgtgctacctgggacgataggatgtactctcccgtgttcggcgggggaacaaagctgactgtcctggagagcaaatatggaccaccatgccctccatgtcctttttgggtcctggtggtcgtgggaggcgtgctggcatgttattccctgctggtcacagtggccttcatcatcttctgggtgcggagcaagcggagccggctgctgcactctgactacatgaacatgaccccccggagacccggccctacaagaaagcattatcagccttacgccccacccagggacttcgcagcttatcgctcccgagtgaaattttctcgcagtgcagatgcccccgcttatcagcagggccagaatcagctgtacaacgagctgaatctggggaggcgcgaggaatacgacgtgctggataagcgacggggccgggaccccgaaatgggaggaaagcctagaaggaaaaacccacaggagggcctgtataatgaactgcagaaggacaaaatggcagaggcctacagcgaaatcggaatgaagggagagcgccgacggggcaaaggacacgatggcctgtatcaggggctgagcaccgccacaaaggacacctacgatgccctgcacatgcaggctctgcctccacgctga

SEQ ID NO: 18 - DNA, 1494 bp, Artificial Sequence
  source: /note="Description of Artificial Sequence: Synthetic polynucleotide"
atgctgctgctggtgacaagcctgctgctgtgcgaactgccccatcccgccttcctgctgattcctgaggtccagctgctggagagcggaggaggactggtgcagcctggaggaagtctgcgactgtcatgcgccgctagcggcttcaccttcagctcctatgcaatgagctgggtgcgacaggcaccaggcaaggggctggagtgggtctccgctatctccggctctggaggctctacttactatgcagacagtgtgaaggggcggttcacaatctccagagataactctaagaacactctgtacctgcagatgaactctctgagagctgaggacaccgcagtgtactattgcgccaagggcaaaaggtactttgattattggggacagggcactatggtgaccgtctctagtggaggaggaggaagcggaggaggaggatccggcggaggaggcagtcagtcagtgctgacacagccacctagcgcctccggaaccccaggacagcgggtcacaatctcttgtagtgggggatcaagcgacattgggagcaacaccgtgaattggtatcagcagctgcctggaacagctccaaagctgctgatctactataacaatcagaggccctccggcgtccctgatcgcttctcaggcagcaaatccgggacttctgcaagtctggccattagtggcctgcagtcagaggacgaagccgattactattgtgctacctgggacgataggatgtactctcccgtgttcggcgggggaacaaagctgactgtcctggagagcaaatatggaccaccatgccctccatgtcctttttgggtcctggtggtcgtgggaggcgtgctggcatgttattccctgctggtcactgtggccttcatcatcttctgggtgcggagcaagcggagccggctgctgcactctgactacatgaacatgactccacggagacccggccctacccggaaacattatcagccctacgccccacccagagattttgccgcttataggtccaagcgcggccgaaagaaactgctgtacatcttcaaacagcccttcatgagacccgtccagacaactcaggaggaagacggctgcagctgtaggttccccgaggaagaggaagggggatgtgagctgagggtgaagttttctcgcagtgcagatgcccctgcttatcagcagggacagaatcagctgtacaacgagctgaatctgggcaggcgcgaggaatacgacgtgctggataagcgacggggcagagaccccgaaatgggagggaagcccagaaggaaaaaccctcaggaggggctgtataatgaactgcagaaggacaaaatggcagaggcctacagtgaaatcgggatgaagggagagcgccgacggggaaaaggccacgatggactgtatcagggcctgtctactgccaccaaggacacctacgatgccctgcacatgcaggctctgcctccacgctga

SEQ ID NO: 19 - protein, 456 aa, Artificial Sequence
  source: /note="Description of Artificial Sequence: Synthetic polypeptide"
MLLLVTSLLLCELPHPAFLLIPDVVMTQSPLSLPVTPGEPASISCRSSQSLVHSNRNTYLHWYLQKPGQSPQLLIYKVSNRFSGVPDRFSGSGSGTDFTLKISRVEAEDVGVYYCSQNTHVPPTFGQGTKLEIKGGGGSGGGGSGGGGSQVQLVQSGAEVKKPGASVKVSCKASGYTFTDYEMHWVRQAPGQGLEWMGALDPKTGDTAYSQKFKGRVTLTADKSTSTAYMELSSLTSEDTAVYYCTRFYSYTYWGQGTLVTVSSDKTHTCPPCPFWVLVVVGGVLACYSLLVTVAFIIFWVKRGRKKLLYIFKQPFMRPVQTTQEEDGCSCRFPEEEEGGCELRVKFSRSADAPAYQQGQNQLYNELNLGRREEYDVLDKRRGRDPEMGGKPQRRKNPQEGLYNELQKDKMAEAYSEIGMKGERRRGKGHDGLYQGLSTATKDTYDALHMQALPPR

SEQ ID NO: 20 - protein, 497 aa, Artificial Sequence
  source: /note="Description of Artificial Sequence: Synthetic polypeptide"
MLLLVTSLLLCELPHPAFLLIPDVVMTQSPLSLPVTPGEPASISCRSSQSLVHSNRNTYLHWYLQKPGQSPQLLIYKVSNRFSGVPDRFSGSGSGTDFTLKISRVEAEDVGVYYCSQNTHVPPTFGQGTKLEIKGGGGSGGGGSGGGGSQVQLVQSGAEVKKPGASVKVSCKASGYTFTDYEMHWVRQAPGQGLEWMGALDPKTGDTAYSQKFKGRVTLTADKSTSTAYMELSSLTSEDTAVYYCTRFYSYTYWGQGTLVTVSSDKTHTCPPCPFWVLVVVGGVLACYSLLVTVAFIIFWVRSKRSRLLHSDYMNMTPRRPGPTRKHYQPYAPPRDFAAYRSKRGRKKLLYIFKQPFMRPVQTTQEEDGCSCRFPEEEEGGCELRVKFSRSADAPAYQQGQNQLYNELNLGRREEYDVLDKRRGRDPEMGGKPQRRKNPQEGLYNELQKDKMAEAYSEIGMKGERRRGKGHDGLYQGLSTATKDTYDALHMQALPPR

SEQ ID NO: 21 - protein, 457 aa, Artificial Sequence
  source: /note="Description of Artificial Sequence: Synthetic polypeptide"
MLLLVTSLLLCELPHPAFLLIPQVQLVQSGGGVVQPGRSLRLSCAASGFTFSSYGLHWVRQAPGKGLEWVAAISYDGSKKYYADSVKGRLTISRDNSKNTLYLQMNSLRPDDTALYFCARGWFVEPLSWGQGTLVTVSSGGGGSGGGGSGGGGSQSVLTQPPSASGTPGQRVTISCSGSSSNIGSNTVNWYQQLPGTAPKLLIYSNNQRPSGVPDRFSGSKSGTSASLAISGLQSEDEADYYCAAWDDSLNGYVFGTGTKLTVLESKYGPPCPPCPFWVLVVVGGVLACYSLLVTVAFIIFWVKRGRKKLLYIFKQPFMRPVQTTQEEDGCSCRFPEEEEGGCELRVKFSRSADAPAYQQGQNQLYNELNLGRREEYDVLDKRRGRDPEMGGKPRRKNPQEGLYNELQKDKMAEAYSEIGMKGERRRGKGHDGLYQGLSTATKDTYDALHMQALPPR

SEQ ID NO: 22 - DNA, 1371 bp, Artificial Sequence
  source: /note="Description of Artificial Sequence: Synthetic polynucleotide"
atgctgctgctggtgacaagcctgctgctgtgcgaactgccccatcccgccttcctgctgattcctgatgtcgtgatgacgcagagccctctctctcttcccgttacccctggtgaacccgcatcaataagttgccgctccagtcaatcacttgtacattcaaatcgcaatacctacctgcactggtatttgcagaagccgggacaatcccctcaattgttgatatataaggtatccaatcgcttttctggagttcctgatagattcagcggatccgggtctggtactgatttcactctgaaaatatccagggtcgaagctgaggacgtaggcgtatattattgctctcagaacacgcatgtcccgccgactttcggccagggcactaaacttgagatcaagggtggggggggcagcggtggtggaggctctggtggaggagggagccaggtccaactcgttcaaagtggcgcagaggtcaaaaagccaggcgcgagcgttaaagtatcatgtaaggccagcggttatactttcactgattatgaaatgcactgggtgcgacaagcccccgggcaaggtcttgagtggatgggtgcacttgatccaaaaactggggatactgcctatagccagaaattcaaagggcgcgtcacactcactgccgacaaaagtacgagcacagcttatatggaattgagttcactgacgagcgaggatacggcagtttattactgtacgcgcttctactcttacacttattgggggcaaggcactttggttactgtgtcctctgacaagacccatacgtgtccaccgtgtcccttctgggtattggttgtggtcggcggtgtccttgcttgttacagccttctcgtgacagtcgcattcataattttttgggtgaaaagaggtcggaaaaagttgctgtatattttcaaacaaccctttatgagacctgtacaaacgactcaggaagaggatggttgtagttgcaggtttccggaggaggaggaaggtgggtgcgaactgcgggtgaaatttagtagaagcgctgacgcaccagcttaccaacaaggacagaaccaattgtacaacgagcttaacttgggtaggagggaggaatatgatgtactggacaaaaggcgaggtcgcgatccggaaatgggaggcaagccacagcgccggaaaaacccgcaggaaggcttgtacaacgaacttcagaaagataaaatggcagaagcatactccgaaatagggatgaaaggtgaacggcggcgaggcaagggccacgacggtctgtaccaagggttgtcaacggcaactaaagacacgtatgatgcacttcatatgcaagctctgccacccaggtga

SEQ ID NO: 23 - DNA, 1494 bp, Artificial Sequence
  source: /note="Description of Artificial Sequence: Synthetic polynucleotide"
atgctgctgctggtgacaagcctgctgctgtgcgaactgccccatcccgccttcctgctgattcctgatgtcgtgatgacgcagagccctctctctcttcccgttacccctggtgaacccgcatcaataagttgccgctccagtcaatcacttgtacattcaaatcgcaatacctacctgcactggtatttgcagaagccgggacaatcccctcaattgttgatatataaggtatccaatcgcttttctggagttcctgatagattcagcggatccgggtctggtactgatttcactctgaaaatatccagggtcgaagctgaggacgtaggcgtatattattgctctcagaacacgcatgtcccgccgactttcggccagggcactaaacttgagatcaagggtggggggggcagcggtggtggaggctctggtggaggagggagccaggtccaactcgttcaaagtggcgcagaggtcaaaaagccaggcgcgagcgttaaagtatcatgtaaggccagcggttatactttcactgattatgaaatgcactgggtgcgacaagcccccgggcaaggtcttgagtggatgggtgcacttgatccaaaaactggggatactgcctatagccagaaattcaaagggcgcgtcacactcactgccgacaaaagtacgagcacagcttatatggaattgagttcactgacgagcgaggatacggcagtttattactgtacgcgcttctactcttacacttattgggggcaaggcactttggttactgtgtcctctgacaagacccatacgtgtccaccgtgtcccttctgggtattggttgtggtcggcggtgtccttgcttgttacagccttctcgtgacagtcgcattcataattttttgggtgcggagcaagcggagccggctgctgcactctgactacatgaacatgactccacggagacccggccctacccggaaacattatcagccctacgccccacccagagattttgccgcttataggtccaaaagaggtcggaaaaagttgctgtatattttcaaacaaccctttatgagacctgtacaaacgactcaggaagaggatggttgtagttgcaggtttccggaggaggaggaaggtgggtgcgaactgcgggtgaaatttagtagaagcgctgacgcaccagcttaccaacaaggacagaaccaattgtacaacgagcttaacttgggtaggagggaggaatatgatgtactggacaaaaggcgaggtcgcgatccggaaatgggaggcaagccacagcgccggaaaaacccgcaggaaggcttgtacaacgaacttcagaaagataaaatggcagaagcatactccgaaatagggatgaaaggtgaacggcggcgaggcaagggccacgacggtctgtaccaagggttgtcaacggcaactaaagacacgtatgatgcacttcatatgcaagctctgccacccaggtga

SEQ ID NO: 24 - DNA, 1374 bp, Artificial Sequence
  source: /note="Description of Artificial Sequence: Synthetic polynucleotide"
atgctgctgctggtgacaagcctgctgctgtgcgaactgccccatcccgccttcctgctgattcctcaggtccagcttgtgcaaagcggaggaggagtggtacagcctggccgctctttgagactgtcttgtgcggccagtggatttacattctcttcttatgggttgcattgggtcagacaagcaccgggcaaaggattggaatgggtcgcggccattagctatgatggctcaaagaaatattatgccgattccgtaaaagggaggttgacaataagccgggataacagcaagaacactttgtatcttcagatgaatagcctccgaccggacgacacggcactgtatttttgcgcacgcgggtggtttgtagaacccctgagttggggacaaggtactcttgtcacggtatcttctggcggaggtgggagtggtgggggtggcagtggcgggggtgggtcacaaagcgtgcttacacaacctccttctgcgagcggaactccgggacaacgggttacgatttcatgctccggctcaagtagcaatataggatcaaatacagtgaattggtatcaacaactccctggcacagcgcccaagctgctgatctactctaataaccagaggccgagtggtgtgccagataggttcagtggctctaaatcaggtactagcgcgagcctcgccatttcaggacttcaatcagaggatgaagcggactactactgtgccgcgtgggatgattcacttaatggatatgttttcgggaccggaacaaaattgacggtattggagagcaaatatggaccaccatgccctccatgtcctttttgggtcctggtggtcgtgggaggcgtgctggcatgttattctctgctggtcacagtggctttcatcatcttctgggtcaagcgaggccggaagaaactgctgtacatcttcaaacagccttttatgcgcccagtgcagacaactcaggaggaagacggctgctcttgtcggttccccgaggaagaggaagggggatgtgagctgcgcgtgaagttttctcgaagtgccgatgctcctgcatatcagcagggacagaaccagctgtacaacgagctgaatctgggccggagagaggaatacgacgtgctggataagaggcgcggcagagacccagaaatgggcgggaagccacgacggaaaaacccccaggaggggctgtataatgaactgcagaaggacaaaatggccgaggcttacagcgaaatcgggatgaagggagagagaaggcgcggaaaaggccacgatggactgtatcagggcctgagcactgccaccaaggacacctacgatgctctgcacatgcaggcactgccacccaggtga

SEQ ID NO: 25 - protein, 456 aa, Artificial Sequence
  source: /note="Description of Artificial Sequence: Synthetic polypeptide"
MLLLVTSLLLCELPHPAFLLIPEVQLLESGGGLVQPGGSLRLSCAASGFTFSSYAMSWVRQAPGKGLEWVSAISGSGGSTYYADSVKGRFTISRDNSKNTLYLQMNSLRAEDTAVYYCARGKRYFDYWGQGTMVTVSSGGGGSGGGGSGGGGSSYELTQPPSASGTPGQRVTISCSGGSSNIGSNTVNWFRQLPGTAPKLLVYFNNQRPSGVPDRFSGSKSGTSASLAIGGLQSDDEADYYCVAWDDSLNAPVFGGGTKVTVLESKYGPPCPPCPFWVLVVVGGVLACYSLLVTVAFIIFWVKRGRKKLLYIFKQPFMRPVQTTQEEDGCSCRFPEEEEGGCELRVKFSRSADAPAYQQGQNQLYNELNLGRREEYDVLDKRRGRDPEMGGKPRRKNPQEGLYNELQKDKMAEAYSEIGMKGERRRGKGHDGLYQGLSTATKDTYDALHMQALPPR

SEQ ID NO: 26 - DNA, 1368 bp, Artificial Sequence
  source: /note="Description of Artificial Sequence: Synthetic polynucleotide"
atgctgctgctggtgacaagcctgctgctgtgcgaactgccccatcccgccttcctgctgattcctgaggtgcagctgttggagtctgggggaggcttggtacagcctggggggtccctgagactctcctgtgcagcctctggattcacctttagcagctatgccatgagctgggtccgccaggctccagggaaggggctggagtgggtctcagctattagtggtagtggtggtagcacatactacgcagactccgtgaagggccggttcaccatctccagagacaattccaagaacacgctgtatctgcaaatgaacagcctgagagccgaggacacggccgtgtattactgtgcgagaggaaagcgatactttgactactggggccaggggacaatggtcaccgtctcgagtggtggggggggcagcggtggtggaggctctggtggaggagggagctcctatgagctgactcagccaccctcagcgtctgggacccccgggcagagggtcaccatctcttgttctggaggcagctccaacatcggaagtaatactgtaaactggttccggcagctcccaggaacggcccccaaactcctcgtttattttaataatcagcgaccctcaggggtccctgaccgattctctggctccaagtctggcacctcggcctccctggccatcggtgggctccagtctgacgatgaggctgactattactgtgtagcatgggatgactctctgaatgctccggtgttcggcggagggaccaaggtcaccgtcctagagagcaaatatggaccaccatgccctccatgtcctttttgggtcctggtggtcgtgggaggcgtgctggcatgttattctctgctggtcacagtggctttcatcatcttctgggtcaagcgaggccggaagaaactgctgtacatcttcaaacagccttttatgcgcccagtgcagacaactcaggaggaagacggctgctcttgtcggttccccgaggaagaggaagggggatgtgagctgcgcgtgaagttttctcgaagtgccgatgctcctgcatatcagcagggacagaaccagctgtacaacgagctgaatctgggccggagagaggaatacgacgtgctggataagaggcgcggcagagacccagaaatgggcgggaagccacgacggaaaaacccccaggaggggctgtataatgaactgcagaaggacaaaatggccgaggcttacagcgaaatcgggatgaagggagagagaaggcgcggaaaaggccacgatggactgtatcagggcctgagcactgccaccaaggacacctacgatgctctgcacatgcaggcactgccacccagg

SEQ ID NO: 27 - protein, 116 aa, Artificial Sequence
  source: /note="Description of Artificial Sequence: Synthetic polypeptide"
EVQLLESGGGLVQPGGSLRLSCAASGFTFSSYAMSWVRQAPGKGLEWVSAISGSGGSTYYADSVKGRFTISRDNSKNTLYLQMNSLRAEDTAVYYCARGKRYFDYWGQGTMVTVSS

SEQ ID NO: 28 - protein, 110 aa, Artificial Sequence
  source: /note="Description of Artificial Sequence: Synthetic polypeptide"
SYELTQPPSASGTPGQRVTISCSGGSSNIGSNTVNWFRQLPGTAPKLLVYFNNQRPSGVPDRFSGSKSGTSASLAIGGLQSDDEADYYCVAWDDSLNAPVFGGGTKVTVL

SEQ ID NO: 29 - protein, 116 aa, Artificial Sequence
  source: /note="Description of Artificial Sequence: Synthetic polypeptide"
EVQLLESGGGLVQPGGSLRLSCAASGFTFSSYAMSWVRQAPGKGLEWVSAISGSGGSTYYADSVKGRFTISRDNSKNTLYLQMNSLRAEDTAVYYCAKGKRYFDYWGQGTMVTVSS

SEQ ID NO: 30 - protein, 110 aa, Artificial Sequence
  source: /note="Description of Artificial Sequence: Synthetic polypeptide"
QSVLTQPPSASGTPGQRVTISCSGGSSDIGSNTVNWYQQLPGTAPKLLIYYNNQRPSGVPDRFSGSKSGTSASLAISGLQSEDEADYYCATWDDRMYSPVFGGGTKLTVL

SEQ ID NO: 31 - protein, 242 aa, Artificial Sequence
  source: /note="Description of Artificial Sequence: Synthetic polypeptide"
DVVMTQSPLSLPVTPGEPASISCRSSQSLVHSNRNTYLHWYLQKPGQSPQLLIYKVSNRFSGVPDRFSGSGSGTDFTLKISRVEAEDVGVYYCSQNTHVPPTFGQGTKLEIKGGGGSGGGGSGGGGSQVQLVQSGAEVKKPGASVKVSCKASGYTFTDYEMHWVRQAPGQGLEWMGALDPKTGDTAYSQKFKGRVTLTADKSTSTAYMELSSLTSEDTAVYYCTRFYSYTYWGQGTLVTVSS

SEQ ID NO: 32 - protein, 242 aa, Artificial Sequence
  source: /note="Description of Artificial Sequence: Synthetic polypeptide"
QVQLVQSGGGVVQPGRSLRLSCAASGFTFSSYGLHWVRQAPGKGLEWVAAISYDGSKKYYADSVKGRLTISRDNSKNTLYLQMNSLRPDDTALYFCARGWFVEPLSWGQGTLVTVSSGGGGSGGGGSGGGGSQSVLTQPPSASGTPGQRVTISCSGSSSNIGSNTVNWYQQLPGTAPKLLIYSNNQRPSGVPDRFSGSKSGTSASLAISGLQSEDEADYYCAAWDDSLNGYVFGTGTKLTVL

SEQ ID NO: 33 - DNA, 723 bp, Artificial Sequence
  source: /note="Description of Artificial Sequence: Synthetic polynucleotide"
gaggtgcagctgttggagtctgggggaggcttggtacagcctggggggtccctgagactctcctgtgcagcctctggattcacctttagcagctatgccatgagctgggtccgccaggctccagggaaggggctggagtgggtctcagctattagtggtagtggtggtagcacatactacgcagactccgtgaagggccggttcaccatctccagagacaattccaagaacacgctgtatctgcaaatgaacagcctgagagccgaggacacggccgtgtattactgtgcgagaggaaagcgatactttgactactggggccaggggacaatggtcaccgtctcgagtggtggggggggcagcggtggtggaggctctggtggaggagggagctcctatgagctgactcagccaccctcagcgtctgggacccccgggcagagggtcaccatctcttgttctggaggcagctccaacatcggaagtaatactgtaaactggttccggcagctcccaggaacggcccccaaactcctcgtttattttaataatcagcgaccctcaggggtccctgaccgattctctggctccaagtctggcacctcggcctccctggccatcggtgggctccagtctgacgatgaggctgactattactgtgtagcatgggatgactctctgaatgctccggtgttcggcggagggaccaaggtcaccgtccta

SEQ ID NO: 34 - DNA, 723 bp, Artificial Sequence
  source: /note="Description of Artificial Sequence: Synthetic polynucleotide"
gaggtccagctgctggagagcggaggaggactggtgcagcctggaggaagtctgcgactgtcatgcgccgctagcggcttcaccttcagctcctatgcaatgagctgggtgcgacaggcaccaggcaaggggctggagtgggtctccgctatctccggctctggaggctctacttactatgcagacagtgtgaaggggcggttcacaatctccagagataactctaagaacactctgtacctgcagatgaactctctgagagctgaggacaccgcagtgtactattgcgccaagggcaaaaggtactttgattattggggacagggcactatggtgaccgtctctagtggaggaggaggaagcggaggaggaggatccggcggaggaggcagtcagtcagtgctgacacagccacctagcgcctccggaaccccaggacagcgggtcacaatctcttgtagtgggggatcaagcgacattgggagcaacaccgtgaattggtatcagcagctgcctggaacagctccaaagctgctgatctactataacaatcagaggccctccggcgtccctgatcgcttctcaggcagcaaatccgggacttctgcaagtctggccattagtggcctgcagtcagaggacgaagccgattactattgtgctacctgggacgataggatgtactctcccgtgttcggcgggggaacaaagctgactgtcctg

SEQ ID NO: 35 - DNA, 726 bp, Artificial Sequence
  source: /note="Description of Artificial Sequence: Synthetic polynucleotide"
gatgtcgtgatgacgcagagccctctctctcttcccgttacccctggtgaacccgcatcaataagttgccgctccagtcaatcacttgtacattcaaatcgcaatacctacctgcactggtatttgcagaagccgggacaatcccctcaattgttgatatataaggtatccaatcgcttttctggagttcctgatagattcagcggatccgggtctggtactgatttcactctgaaaatatccagggtcgaagctgaggacgtaggcgtatattattgctctcagaacacgcatgtcccgccgactttcggccagggcactaaacttgagatcaagggtggggggggcagcggtggtggaggctctggtggaggagggagccaggtccaactcgttcaaagtggcgcagaggtcaaaaagccaggcgcgagcgttaaagtatcatgtaaggccagcggttatactttcactgattatgaaatgcactgggtgcgacaagcccccgggcaaggtcttgagtggatgggtgcacttgatccaaaaactggggatactgcctatagccagaaattcaaagggcgcgtcacactcactgccgacaaaagtacgagcacagcttatatggaattgagttcactgacgagcgaggatacggcagtttattactgtacgcgcttctactcttacacttattgggggcaaggcactttggttactgtgtcctct

SEQ ID NO: 36 - DNA, 726 bp, Artificial Sequence
  source: /note="Description of Artificial Sequence: Synthetic polynucleotide"
caggtccagcttgtgcaaagcggaggaggagtggtacagcctggccgctctttgagactgtcttgtgcggccagtggatttacattctcttcttatgggttgcattgggtcagacaagcaccgggcaaaggattggaatgggtcgcggccattagctatgatggctcaaagaaatattatgccgattccgtaaaagggaggttgacaataagccgggataacagcaagaacactttgtatcttcagatgaatagcctccgaccggacgacacggcactgtatttttgcgcacgcgggtggtttgtagaacccctgagttggggacaaggtactcttgtcacggtatcttctggcggaggtgggagtggtgggggtggcagtggcgggggtgggtcacaaagcgtgcttacacaacctccttctgcgagcggaactccgggacaacgggttacgatttcatgctccggctcaagtagcaatataggatcaaatacagtgaattggtatcaacaactccctggcacagcgcccaagctgctgatctactctaataaccagaggccgagtggtgtgccagataggttcagtggctctaaatcaggtactagcgcgagcctcgccatttcaggacttcaatcagaggatgaagcggactactactgtgccgcgtgggatgattcacttaatggatatgttttcgggaccggaacaaaattgacggtattg

SEQ ID NO: 37 - protein, 10 aa, Artificial Sequence
  source: /note="Description of Artificial Sequence: Synthetic peptide"
GFTFSSYAMS

SEQ ID NO: 38 - protein, 17 aa, Artificial Sequence
  source: /note="Description of Artificial Sequence: Synthetic peptide"
AISGSGGSTYYADSVKG

SEQ ID NO: 39 - protein, 7 aa, Artificial Sequence
  source: /note="Description of Artificial Sequence: Synthetic peptide"
GKRYFDY

SEQ ID NO: 40 - protein, 13 aa, Artificial Sequence
  source: /note="Description of Artificial Sequence: Synthetic peptide"
SGGSSNIGSNTVN

SEQ ID NO: 41 - protein, 7 aa, Artificial Sequence
  source: /note="Description of Artificial Sequence: Synthetic peptide"
FNNQRPS

SEQ ID NO: 42 - protein, 11 aa, Artificial Sequence
  source: /note="Description of Artificial Sequence: Synthetic peptide"
VAWDDSLNAPV

SEQ ID NO: 43 - protein, 13 aa, Artificial Sequence
  source: /note="Description of Artificial Sequence: Synthetic peptide"
SGGSSDIGSNTVN

SEQ ID NO: 44 - protein, 7 aa, Artificial Sequence
  source: /note="Description of Artificial Sequence: Synthetic peptide"
YNNQRPS

SEQ ID NO: 45 - protein, 11 aa, Artificial Sequence
  source: /note="Description of Artificial Sequence: Synthetic peptide"
ATWDDRMYSPV

SEQ ID NO: 46 - DNA, 2013 bp, Artificial Sequence
  source: /note="Description of Artificial Sequence: Synthetic polynucleotide"
atgctgctgctggtgacaagcctgctgctgtgcgaactgccccatcccgccttcctgctgattcctgaggtgcagctgttggagtctgggggaggcttggtacagcctggggggtccctgagactctcctgtgcagcctctggattcacctttagcagctatgccatgagctgggtccgccaggctccagggaaggggctggagtgggtctcagctattagtggtagtggtggtagcacatactacgcagactccgtgaagggccggttcaccatctccagagacaattccaagaacacgctgtatctgcaaatgaacagcctgagagccgaggacacggccgtgtattactgtgcgagaggaaagcgatactttgactactggggccaggggacaatggtcaccgtctcgagtggtggggggggcagcggtggtggaggctctggtggaggagggagctcctatgagctgactcagccaccctcagcgtctgggacccccgggcagagggtcaccatctcttgttctggaggcagctccaacatcggaagtaatactgtaaactggttccggcagctcccaggaacggcccccaaactcctcgtttattttaataatcagcgaccctcaggggtccctgaccgattctctggctccaagtctggcacctcggcctccctggccatcggtgggctccagtctgacgatgaggctgactattactgtgtagcatgggatgactctctgaatgctccggtgttcggcggagggaccaaggtcaccgtcctagagagcaaatatggaccaccatgccctccatgtcctttttgggtcctggtggtcgtgggaggcgtgctggcatgttattctctgctggtcacagtggctttcatcatcttctgggtcaagcgaggccggaagaaactgctgtacatcttcaaacagccttttatgcgcccagtgcagacaactcaggaggaagacggctgctcttgtcggttccccgaggaagaggaagggggatgtgagctgcgcgtgaagttttctcgaagtgccgatgctcctgcatatcagcagggacagaaccagctgtacaacgagctgaatctgggccggagagaggaatacgacgtgctggataagaggcgcggcagagacccagaaatgggcgggaagccacgacggaaaaacccccaggaggggctgtataatgaactgcagaaggacaaaatggccgaggcttacagcgaaatcgggatgaagggagagagaaggcgcggaaaaggccacgatggactgtatcagggcctgagcactgccaccaaggacacctacgatgctctgcacatgcaggcactgccacccaggggtagcggcgagggcagaggaagtcttctaacatgcggtgacgtggaggagaatcccggccctatgggtcgggggctgctcaggggcctgtggccgctgcacatcgtcctgtggacgcgtatcgccagcacgatcccaccgcacgttcagaagtcggttaataacgacatgatagtcactgacaacaacggtgcagtcaagtttccacaactgtgtaaattttgtgatgtgagattttccacctgtgacaaccagaaatcctgcatgagcaactgcagcatcacctccatctgtgagaagccacaggaagtctgtgtggctgtatggagaaagaatgacgagaacataacactagagacagtttgccatgaccccaagctcccctaccatgactttattctggaagatgctgcttctccaaagtgcattatgaaggaaaaaaaaaagcctggtgagactttcttcatgtgttcctgtagctctgatgagtgcaatgacaacatcatcttctcagaagaatataacaccagcaatcctgacttgttgctagtcatatttcaagtgacaggcatcagcctcctgccaccactgggagttgccatatctgtcatcatcatcttctactgctaccgcgttaaccggcag

SEQ ID NO: 47 - protein, 671 aa, Artificial Sequence
  source: /note="Description of Artificial Sequence: Synthetic polypeptide"
MLLLVTSLLLCELPHPAFLLIPEVQLLESGGGLVQPGGSLRLSCAASGFTFSSYAMSWVRQAPGKGLEWVSAISGSGGSTYYADSVKGRFTISRDNSKNTLYLQMNSLRAEDTAVYYCARGKRYFDYWGQGTMVTVSSGGGGSGGGGSGGGGSSYELTQPPSASGTPGQRVTISCSGGSSNIGSNTVNWFRQLPGTAPKLLVYFNNQRPSGVPDRFSGSKSGTSASLAIGGLQSDDEADYYCVAWDDSLNAPVFGGGTKVTVLESKYGPPCPPCPFWVLVVVGGVLACYSLLVTVAFIIFWVKRGRKKLLYIFKQPFMRPVQTTQEEDGCSCRFPEEEEGGCELRVKFSRSADAPAYQQGQNQLYNELNLGRREEYDVLDKRRGRDPEMGGKPRRKNPQEGLYNELQKDKMAEAYSEIGMKGERRRGKGHDGLYQGLSTATKDTYDALHMQALPPRGSGEGRGSLLTCGDVEENPGPMGRGLLRGLWPLHIVLWTRIASTIPPHVQKSVNNDMIVTDNNGAVKFPQLCKFCDVRFSTCDNQKSCMSNCSITSICEKPQEVCVAVWRKNDENITLETVCHDPKLPYHDFILEDAASPKCIMKEKKKPGETFFMCSCSSDECNDNIIFSEEYNTSNPDLLLVIFQVTGISLLPPLGVAISVIIIFYCYRVNRQ

SEQ ID NO: 48 - protein, 15 aa, Artificial Sequence
  source: /note="Description of Artificial Sequence: Synthetic peptide"
  SITE (1)..(15): /note="This sequence may encompass 1-3 'Gly Gly Gly Gly Ser' repeating units"
  source: /note="See specification as filed for detailed description of substitutions and preferred embodiments"
GGGGSGGGGSGGGGS